European Patent Application EP 4 397 679 A1, published July 10, 2024. Title: ENGINEERED TGFΒRII VARIANTS AND METHODS OF USE THEREOF. Applicant: FBD Biologics Limited. Application EP. The sequence listing filed with the application follows.

SEQUENCE LISTING (17 sequences)

SEQ ID NO: 1 - protein, 386 aa, synthetic construct
ESKYGPPCPPCPAPEFLGGPSVFLFPPKPKDTLMISRTPEVTCVVVDVSQEDPEVQFNWYVDGVEVHNAKTKPREEQFNSTYRVVSVLTVLHQDWLNGKEYKCKVSNKGLPSSIEKTISKAKGQPREPQVYTLPPSQEEMTKNQVSLTCLVKGFYPSDIAVEWESNGQPENNYKTTPPVLDSDGSFFLYSRLTVDKSRWQEGNVFSCSVMHEALHNHYTQKSLSLSLGAGGGGSGGGGSGGGGSGGGGSGIPPHVQKSVNNDMIVTDNNGAVKFPQLCKFCDVRFSTCDNQKSCMSNCSITSICEKPQEVCVAVWRKNDENITLETVCHDPKLPYHDFILEDAASPKCIMKEKKKPGETFFMCSCSSDECNDNIIFSEEYNTSNPD

SEQ ID NO: 2 - protein, 386 aa, synthetic construct
ESKYGPPCPPCPAPEFLGGPSVFLFPPKPKDTLMISRTPEVTCVVVDVSQEDPEVQFNWYVDGVEVHNAKTKPREEQFNSTYRVVSVLTVLHQDWLNGKEYKCKVSNKGLPSSIEKTISKAKGQPREPQVYTLPPSQEEMTKNQVSLTCLVKGFYPSDIAVEWESNGQPENNYKTTPPVLDSDGSFFLYSRLTVDKSRWQEGNVFSCSVMHEALHNHYTQKSLSLSLGAGGGGSGGGGSGGGGSGGGGSGIPPHVQKSVNNDMIVTDNNGAVKFPQLCKFCDVRFSTCDNQKSCMSNCEITSICEKPQEVCVAVWRKNDENITLETVCHDPKLPYHDFILEDAASPKCIMKEKKKPGETFFMCSCSSDECNDNIIFSEEYNTSNPD

SEQ ID NO: 3 - protein, 386 aa, synthetic construct
ESKYGPPCPPCPAPEFLGGPSVFLFPPKPKDTLMISRTPEVTCVVVDVSQEDPEVQFNWYVDGVEVHNAKTKPREEQFNSTYRVVSVLTVLHQDWLNGKEYKCKVSNKGLPSSIEKTISKAKGQPREPQVYTLPPSQEEMTKNQVSLTCLVKGFYPSDIAVEWESNGQPENNYKTTPPVLDSDGSFFLYSRLTVDKSRWQEGNVFSCSVMHEALHNHYTQKSLSLSLGAGGGGSGGGGSGGGGSGGGGSGIPPHVQKSVNNDMIVTDNNGAVKFPQLCKFCDVRFSTCDNQKSCMSNCQITSICEKPQEVCVAVWRKNDENITLETVCHDPKLPYHDFILEDAASPKCIMKEKKKPGETFFMCSCSSDECNDNIIFSEEYNTSNPD

SEQ ID NO: 4 - protein, 386 aa, synthetic construct
ESKYGPPCPPCPAPEFLGGPSVFLFPPKPKDTLMISRTPEVTCVVVDVSQEDPEVQFNWYVDGVEVHNAKTKPREEQFNSTYRVVSVLTVLHQDWLNGKEYKCKVSNKGLPSSIEKTISKAKGQPREPQVYTLPPSQEEMTKNQVSLTCLVKGFYPSDIAVEWESNGQPENNYKTTPPVLDSDGSFFLYSRLTVDKSRWQEGNVFSCSVMHEALHNHYTQKSLSLSLGAGGGGSGGGGSGGGGSGGGGSGIPPHVQKSVNNDMIVTDNNGAVKFPQLCKFCDVRFSTCDNQKSCMSNCSITSICEKPQEVCVAVWRKNDENITLETVCHDPKLPYHDFILEDAASPKCIMKEKKKPGETFFMCSCSSEECNDNIIFSEEYNTSNPD

SEQ ID NO: 5 - protein, 386 aa, synthetic construct
ESKYGPPCPPCPAPEFLGGPSVFLFPPKPKDTLMISRTPEVTCVVVDVSQEDPEVQFNWYVDGVEVHNAKTKPREEQFNSTYRVVSVLTVLHQDWLNGKEYKCKVSNKGLPSSIEKTISKAKGQPREPQVYTLPPSQEEMTKNQVSLTCLVKGFYPSDIAVEWESNGQPENNYKTTPPVLDSDGSFFLYSRLTVDKSRWQEGNVFSCSVMHEALHNHYTQKSLSLSLGAGGGGSGGGGSGGGGSGGGGSGIPPHVQKSVNNDMIVTDNNGAVKFPQLCKFCDVRFSTCDNQKSCMSNCEITSICEKPQEVCVAVWRKNDENITLETVCHDPKLPYHDFILEDAASPKCIMKEKKKPGETFFMCSCSSEECNDNIIFSEEYNTSNPD

SEQ ID NO: 6 - protein, 386 aa, synthetic construct
ESKYGPPCPPCPAPEFLGGPSVFLFPPKPKDTLMISRTPEVTCVVVDVSQEDPEVQFNWYVDGVEVHNAKTKPREEQFNSTYRVVSVLTVLHQDWLNGKEYKCKVSNKGLPSSIEKTISKAKGQPREPQVYTLPPSQEEMTKNQVSLTCLVKGFYPSDIAVEWESNGQPENNYKTTPPVLDSDGSFFLYSRLTVDKSRWQEGNVFSCSVMHEALHNHYTQKSLSLSLGAGGGGSGGGGSGGGGSGGGGSGIPPHVQKSVNNDMIVTDNNGAVKFPQLCKFCDVRFSTCDNQKSCMSNCQITSICEKPQEVCVAVWRKNDENITLETVCHDPKLPYHDFILEDAASPKCIMKEKKKPGETFFMCSCSSEECNDNIIFSEEYNTSNPD

SEQ ID NO: 7 - protein, 136 aa, Homo sapiens
IPPHVQKSVNNDMIVTDNNGAVKFPQLCKFCDVRFSTCDNQKSCMSNCSITSICEKPQEVCVAVWRKNDENITLETVCHDPKLPYHDFILEDAASPKCIMKEKKKPGETFFMCSCSSDECNDNIIFSEEYNTSNPD

SEQ ID NO: 8 - protein, 136 aa, synthetic construct
IPPHVQKSVNNDMIVTDNNGAVKFPQLCKFCDVRFSTCDNQKSCMSNCEITSICEKPQEVCVAVWRKNDENITLETVCHDPKLPYHDFILEDAASPKCIMKEKKKPGETFFMCSCSSDECNDNIIFSEEYNTSNPD

SEQ ID NO: 9 - protein, 136 aa, synthetic construct
IPPHVQKSVNNDMIVTDNNGAVKFPQLCKFCDVRFSTCDNQKSCMSNCQITSICEKPQEVCVAVWRKNDENITLETVCHDPKLPYHDFILEDAASPKCIMKEKKKPGETFFMCSCSSDECNDNIIFSEEYNTSNPD

SEQ ID NO: 10 - protein, 136 aa, synthetic construct
IPPHVQKSVNNDMTVTDNNGAVKFPQLCKFCDVRFSTCDNQKSCMSNCSTTSTCEKPQEVCVAVWRKNDENTTLETVCHDPKLPYHDFTLEDAASPKCTMKEKKKPGETFFMCSCSSEECNDNTTFSEEYNTSNPD

SEQ ID NO: 11 - protein, 136 aa, synthetic construct
IPPHVQKSVNNDMTVTDNNGAVKFPQLCKFCDVRFSTCDNQKSCMSNCETTSTCEKPQEVCVAVWRKNDENTTLETVCHDPKLPYHDFTLEDAASPKCTMKEKKKPGETFFMCSCSSEECNDNTTFSEEYNTSNPD

SEQ ID NO: 12 - protein, 136 aa, synthetic construct
IPPHVQKSVNNDMTVTDNNGAVKFPQLCKFCDVRFSTCDNQKSCMSNCQTTSTCEKPQEVCVAVWRKNDENTTLETVCHDPKLPYHDFTLEDAASPKCTMKEKKKPGETFFMCSCSSEECNDNTTFSEEYNTSNPD

SEQ ID NO: 13 - protein, 228 aa, synthetic construct
ESKYGPPCPPCPAPEFLGGPSVFLFPPKPKDTLMTSRTPEVTCVVVDVSQEDPEVQFNWYVDGVEVHNAKTKPREEQFNSTYRVVSVLTVLHQDWLNGKEYKCKVSNKGLPSSTEKTTSKAKGQPREPQVYTLPPSQEEMTKNQVSLTCLVKGFYPSDTAVEWESNGQPENNYKTTPPVLDSDGSFFLYSRLTVDKSRWQEGNVFSCSVMHEALHNHYTQKSLSLSLG

SEQ ID NO: 14 - protein, 20 aa, synthetic construct
GGGGSGGGGSGGGGSGGGGS

SEQ ID NO: 15 - protein, 112 aa, Homo sapiens
ALDTNYCFSSTEKNCCVRQLYIDFRKDLGWKWIHEPKGYHANFCLGPCPYIWSLDTQYSKVLALYNQHNPGASAAPCCVPQALEPLPIVYYVGRKPKVEQLSNMIVRSCKCS

SEQ ID NO: 16 - protein, 112 aa, Homo sapiens
ALDAAYCFRNVQDNCCLRPLYIDFKRDLGWKWIHEPKGYNANFCAGACPYLWSSDTQHSRVLSLYNTINPEASASPCCVSQDLEPLTILYYIGKTPKIEQLSNMIVKSCKCS

SEQ ID NO: 17 - protein, 112 aa, Homo sapiens; identical to SEQ ID NO: 15